European Patent Application EP 4 119 577 A2, published January 18, 2023. Title: Compositions and Methods of Inhibiting MASP-1 and/or MASP-2 and/or MASP-3 for the Treatment of Various Diseases and Disorders. Applicant: Omeros Corporation University of Leicester. The sequence listing filed with the application follows.

SEQUENCE LISTING (42 sequences)

SEQ ID NO: 1 - DNA, 725 bp, homo sapiens
ggccaggccagctggacgggcacaccatgaggctgctgaccctcctgggccttctgtgtggctcggtggccacccccttgggcccgaagtggcctgaacctgtgttcgggcgcctggcatcccccggctttccaggggagtatgccaatgaccaggagcggcgctggaccctgactgcaccccccggctaccgcctgcgcctctacttcacccacttcgacctggagctctcccacctctgcgagtacgacttcgtcaagctgagctcgggggccaaggtgctggccacgctgtgcgggcaggagagcacagacacggagcgggcccctggcaaggacactttctactcgctgggctccagcctggacattaccttccgctccgactactccaacgagaagccgttcacggggttcgaggccttctatgcagccgaggacattgacgagtgccaggtggccccgggagaggcgcccacctgcgaccaccactgccacaaccacctgggcggtttctactgctcctgccgcgcaggctacgtcctgcaccgtaacaagcgcacctgctcagagcagagcctctagcctcccctggagctccggcctgcccagcaggtcagaagccagagccagcctgctggcctcagctccgggttgggctgagatggctgtgccccaactcccattcacccaccatggacccaataataaacctggccccacccc

SEQ ID NO: 2 - protein, 185 aa, homo sapiens
MRLLTLLGLLCGSVATPLGPKWPEPVFGRLASPGFPGEYANDQERRWTLTAPPGYRLRLYFTHFDLELSHLCEYDFVKLSSGAKVLATLCGQESTDTERAPGKDTFYSLGSSLDITFRSDYSNEKPFTGFEAFYAAEDIDECQVAPGEAPTCDHHCHNHLGGFYCSCRAGYVLHRNKRTCSEQSL

SEQ ID NO: 3 - protein, 170 aa, homo sapiens
TPLGPKWPEPVFGRLASPGFPGEYANDQERRWTLTAPPGYRLRLYFTHFDLELSHLCEYDFVKLSSGAKVLATLCGQESTDTERAPGKDTFYSLGSSLDITFRSDYSNEKPFTGFEAFYAAEDIDECQVAPGEAPTCDHHCHNHLGGFYCSCRAGYVLHRNKRTCSEQSL

SEQ ID NO: 4 - DNA, 2460 bp, homo sapiens
ggccagctggacgggcacaccatgaggctgctgaccctcctgggccttctgtgtggctcggtggccacccccttgggcccgaagtggcctgaacctgtgttcgggcgcctggcatcccccggctttccaggggagtatgccaatgaccaggagcggcgctggaccctgactgcaccccccggctaccgcctgcgcctctacttcacccacttcgacctggagctctcccacctctgcgagtacgacttcgtcaagctgagctcgggggccaaggtgctggccacgctgtgcgggcaggagagcacagacacggagcgggcccctggcaaggacactttctactcgctgggctccagcctggacattaccttccgctccgactactccaacgagaagccgttcacggggttcgaggccttctatgcagccgaggacattgacgagtgccaggtggccccgggagaggcgcccacctgcgaccaccactgccacaaccacctgggcggtttctactgctcctgccgcgcaggctacgtcctgcaccgtaacaagcgcacctgctcagccctgtgctccggccaggtcttcacccagaggtctggggagctcagcagccctgaatacccacggccgtatcccaaactctccagttgcacttacagcatcagcctggaggaggggttcagtgtcattctggactttgtggagtccttcgatgtggagacacaccctgaaaccctgtgtccctacgactttctcaagattcaaacagacagagaagaacatggcccattctgtgggaagacattgccccacaggattgaaacaaaaagcaacacggtgaccatcacctttgtcacagatgaatcaggagaccacacaggctggaagatccactacacgagcacagcgcagccttgcccttatccgatggcgccacctaatggccacgtttcacctgtgcaagccaaatacatcctgaaagacagcttctccatcttttgcgagactggctatgagcttctgcaaggtcacttgcccctgaaatcctttactgcagtttgtcagaaagatggatcttgggaccggccaatgcccgcgtgcagcattgttgactgtggccctcctgatgatctacccagtggccgagtggagtacatcacaggtcctggagtgaccacctacaaagctgtgattcagtacagctgtgaagagaccttctacacaatgaaagtgaatgatggtaaatatgtgtgtgaggctgatggattctggacgagctccaaaggagaaaaatcactcccagtctgtgagcctgtttgtggactatcagcccgcacaacaggagggcgtatatatggagggcaaaaggcaaaacctggtgattttccttggcaagtcctgatattaggtggaaccacagcagcaggtgcacttttatatgacaactgggtcctaacagctgctcatgccgtctatgagcaaaaacatgatgcatccgccctggacattcgaatgggcaccctgaaaagactatcacctcattatacacaagcctggtctgaagctgtttttatacatgaaggttatactcatgatgctggctttgacaatgacatagcactgattaaattgaataacaaagttgtaatcaatagcaacatcacgcctatttgtctgccaagaaaagaagctgaatcctttatgaggacagatgacattggaactgcatctggatggggattaacccaaaggggttttcttgctagaaatctaatgtatgtcgacataccgattgttgaccatcaaaaatgtactgctgcatatgaaaagccaccctatccaaggggaagtgtaactgctaacatgctttgtgctggcttagaaagtgggggcaaggacagctgcagaggtgacagcggaggggcactggtgtttctagatagtgaaacagagaggtggtttgtgggaggaatagtgtcctggggttccatgaattgtggggaagcaggtcagtatggagtctacacaaaagttattaactatattccctggatcgagaacataattagtgatttttaacttgcgtgtctgcagtcaaggattcttcatttttagaaatgcctgtgaagaccttggcagcgacgtggctcgagaagcattcatcattactgtggacatggcagttgttgctccacccaaaaaaacagactccaggtgaggctgctgtcatttctccacttgccagtttaattccagccttacccattgactcaaggggacataaaccacgagagtgacagtcatctttgcccacccagtgtaatgtcactgctcaaattacatttcattaccttaaaaagccagtctcttttcatactggctgttggcatttctgtaaactgcctgtccatgctctttgtttttaaacttgttcttattgaaaaaaaaaaaaaaaaa

SEQ ID NO: 5 - protein, 686 aa, homo sapiens
MRLLTLLGLLCGSVATPLGPKWPEPVFGRLASPGFPGEYANDQERRWTLTAPPGYRLRLYFTHFDLELSHLCEYDFVKLSSGAKVLATLCGQESTDTERAPGKDTFYSLGSSLDITFRSDYSNEKPFTGFEAFYAAEDIDECQVAPGEAPTCDHHCHNHLGGFYCSCRAGYVLHRNKRTCSALCSGQVFTQRSGELSSPEYPRPYPKLSSCTYSISLEEGFSVILDFVESFDVETHPETLCPYDFLKIQTDREEHGPFCGKTLPHRIETKSNTVTITFVTDESGDHTGWKIHYTSTAQPCPYPMAPPNGHVSPVQAKYILKDSFSIFCETGYELLQGHLPLKSFTAVCQKDGSWDRPMPACSIVDCGPPDDLPSGRVEYITGPGVTTYKAVIQYSCEETFYTMKVNDGKYVCEADGFWTSSKGEKSLPVCEPVCGLSARTTGGRIYGGQKAKPGDFPWQVLILGGTTAAGALLYDNWVLTAAHAVYEQKHDASALDIRMGTLKRLSPHYTQAWSEAVFIHEGYTHDAGFDNDIALIKLNNKVVINSNITPICLPRKEAESFMRTDDIGTASGWGLTQRGFLARNLMYVDIPIVDHQKCTAAYEKPPYPRGSVTANMLCAGLESGGKDSCRGDSGGALVFLDSETERWFVGGIVSWGSMNCGEAGQYGVYTKVINYIPWIENIISDF

SEQ ID NO: 6 - protein, 671 aa, homo sapiens
TPLGPKWPEPVFGRLASPGFPGEYANDQERRWTLTAPPGYRLRLYFTHFDLELSHLCEYDFVKLSSGAKVLATLCGQESTDTERAPGKDTFYSLGSSLDITFRSDYSNEKPFTGFEAFYAAEDIDECQVAPGEAPTCDHHCHNHLGGFYCSCRAGYVLHRNKRTCSALCSGQVFTQRSGELSSPEYPRPYPKLSSCTYSISLEEGFSVILDFVESFDVETHPETLCPYDFLKIQTDREEHGPFCGKTLPHRIETKSNTVTITFVTDESGDHTGWKIHYTSTAQPCPYPMAPPNGHVSPVQAKYILKDSFSIFCETGYELLQGHLPLKSFTAVCQKDGSWDRPMPACSIVDCGPPDDLPSGRVEYITGPGVTTYKAVIQYSCEETFYTMKVNDGKYVCEADGFWTSSKGEKSLPVCEPVCGLSARTTGGRIYGGQKAKPGDFPWQVLILGGTTAAGALLYDNWVLTAAHAVYEQKHDASALDIRMGTLKRLSPHYTQAWSEAVFIHEGYTHDAGFDNDIALIKLNNKVVINSNITPICLPRKEAESFMRTDDIGTASGWGLTQRGFLARNLMYVDIPIVDHQKCTAAYEKPPYPRGSVTANMLCAGLESGGKDSCRGDSGGALVFLDSETERWFVGGIVSWGSMNCGEAGQYGVYTKVINYIPWIENIISDF

SEQ ID NO: 7 - DNA, 3895 bp, homo sapiens
attccggcacagggacacaaacaagctcacccaacaaagccaagctgggaggaccaaggccgggcagccgggagcacccaaggcaggaaaatgaggtggctgcttctctattatgctctgtgcttctccctgtcaaaggcttcagcccacaccgtggagctaaacaatatgtttggccagatccagtcgcctggttatccagactcctatcccagtgattcagaggtgacttggaatatcactgtcccagatgggtttcggatcaagctttacttcatgcacttcaacttggaatcctcctacctttgtgaatatgactatgtgaaggtagaaactgaggaccaggtgctggcaaccttctgtggcagggagaccacagacacagagcagactcccggccaggaggtggtcctctcccctggctccttcatgtccatcactttccggtcagatttctccaatgaggagcgtttcacaggctttgatgcccactacatggctgtggatgtggacgagtgcaaggagagggaggacgaggagctgtcctgtgaccactactgccacaactacattggcggctactactgctcctgccgcttcggctacatcctccacacagacaacaggacctgccgagtggagtgcagtgacaacctcttcactcaaaggactggggtgatcaccagccctgacttcccaaacccttaccccaagagctctgaatgcctgtataccatcgagctggaggagggtttcatggtcaacctgcagtttgaggacatatttgacattgaggaccatcctgaggtgccctgcccctatgactacatcaagatcaaagttggtccaaaagttttggggcctttctgtggagagaaagccccagaacccatcagcacccagagccacagtgtcctgatcctgttccatagtgacaactcgggagagaaccggggctggaggctctcatacagggctgcaggaaatgagtgcccagagctacagcctcctgtccatgggaaaatcgagccctcccaagccaagtatttcttcaaagaccaagtgctcgtcagctgtgacacaggctacaaagtgctgaaggataatgtggagatggacacattccagattgagtgtctgaaggatgggacgtggagtaacaagattcccacctgtaaaattgtagactgtagagccccaggagagctggaacacgggctgatcaccttctctacaaggaacaacctcaccacatacaagtctgagatcaaatactcctgtcaggagccctattacaagatgctcaacaataacacaggtatatatacctgttctgcccaaggagtctggatgaataaagtattggggagaagcctacccacctgccttccagagtgtggtcagccctcccgctccctgccaagcctggtcaagaggatcattgggggccgaaatgctgagcctggcctcttcccgtggcaggccctgatagtggtggaggacacttcgagagtgccaaatgacaagtggtttgggagtggggccctgctctctgcgtcctggatcctcacagcagctcatgtgctgcgctcccagcgtagagacaccacggtgataccagtctccaaggagcatgtcaccgtctacctgggcttgcatgatgtgcgagacaaatcgggggcagtcaacagctcagctgcccgagtggtgctccacccagacttcaacatccaaaactacaaccacgatatagctctggtgcagctgcaggagcctgtgcccctgggaccccacgttatgcctgtctgcctgccaaggcttgagcctgaaggcccggccccccacatgctgggcctggtggccggctggggcatctccaatcccaatgtgacagtggatgagatcatcagcagtggcacacggaccttgtcagatgtcctgcagtatgtcaagttacccgtggtgcctcacgctgagtgcaaaactagctatgagtcccgctcgggcaattacagcgtcacggagaacatgttctgtgctggctactacgagggcggcaaagacacgtgccttggagatagcggtggggcctttgtcatctttgatgacttgagccagcgctgggtggtgcaaggcctggtgtcctgggggggacctgaagaatgcggcagcaagcaggtctatggagtctacacaaaggtctccaattacgtggactgggtgtgggagcagatgggcttaccacaaagtgttgtggagccccaggtggaacggtgagctgacttacttcctcggggcctgcctcccctgagcgaagctacaccgcacttccgacagcacactccacattacttatcagaccatatggaatggaacacactgacctagcggtggcttctcctaccgagacagcccccaggaccctgagaggcagagtgtggtatagggaaaaggctccaggcaggagacctgtgttcctgagcttgtccaagtctctttccctgtctgggcctcactctaccgagtaatacaatgcaggagctcaaccaaggcctctgtgccaatcccagcactcctttccaggccatgcttcttaccccagtggcctttattcactcctgaccacttatcaaacccatcggtcctactgttggtataactgagcttggacctgactattagaaaatggtttctaacattgaactgaatgccgcatctgtatattttcctgctctgccttctgggactagccttggcctaatccttcctctaggagaagagcattcaggttttgggagatggctcatagccaagcccctctctcttagtgtgatcccttggagcaccttcatgcctggggtttctctcccaaaagcttcttgcagtctaagccttatcccttatgttccccattaaaggaatttcaaaagacatggagaaagttgggaaggtttgtgctgactgctgggagcagaatagccgtgggaggcccaccaagcccttaaattcccattgtcaactcagaacacatttgggcccatatgccaccctggaacaccagctgacaccatgggcgtccacacctgctgctccagacaagcacaaagcaatctttcagccttgaaatgtattatctgaaaggctacctgaagcccaggcccgaatatggggacttagtcgattacctggaaaaagaaaagacccacactgtgtcctgctgtgcttttgggcaggaaaatggaagaaagagtggggtgggcacattagaagtcacccaaatcctgccaggctgcctggcatccctggggcatgagctgggcggagaatccaccccgcaggatgttcagagggacccactccttcatttttcagagtcaaaggaatcagaggctcacccatggcaggcagtgaaaagagccaggagtcctgggttctagtccctgctctgcccccaactggctgtataacctttgaaaaatcattttctttgtctgagtctctggttctccgtcagcaacaggctggcataaggtcccctgcaggttccttctagctggagcactcagagcttccctgactgctagcagcctctctggccctcacagggctgattgttctccttctccctggagctctctctcctgaaaatctccatcagagcaaggcagccagagaagcccctgagagggaatgattgggaagtgtccactttctcaaccggctcatcaaacacactcctttgtctatgaatggcacatgtaaatgatgttatattttgtatcttttatatcatatgcttcaccattctgtaaagggcctctgcattgttgctcccatcaggggtctcaagtggaaataaaccctcgtggataaccaaaaaaaaaaaaaaaaaaaa

SEQ ID NO: 8 - protein, 728 aa, homo sapiens
MRWLLLYYALCFSLSKASAHTVELNNMFGQIQSPGYPDSYPSDSEVTWNITVPDGFRIKLYFMHFNLESSYLCEYDYVKVETEDQVLATFCGRETTDTEQTPGQEVVLSPGSFMSITFRSDFSNEERFTGFDAHYMAVDVDECKEREDEELSCDHYCHNYIGGYYCSCRFGYILHTDNRTCRVECSDNLFTQRTGVITSPDFPNPYPKSSECLYTIELEEGFMVNLQFEDIFDIEDHPEVPCPYDYIKIKVGPKVLGPFCGEKAPEPISTQSHSVLILFHSDNSGENRGWRLSYRAAGNECPELQPPVHGKIEPSQAKYFFKDQVLVSCDTGYKVLKDNVEMDTFQIECLKDGTWSNKIPTCKIVDCRAPGELEHGLITFSTRNNLTTYKSEIKYSCQEPYYKMLNNNTGIYTCSAQGVWMNKVLGRSLPTCLPECGQPSRSLPSLVKRIIGGRNAEPGLFPWQALIVVEDTSRVPNDKWFGSGALLSASWILTAAHVLRSQRRDTTVIPVSKEHVTVYLGLHDVRDKSGAVNSSAARVVLHPDFNIQNYNHDIALVQLQEPVPLGPHVMPVCLPRLEPEGPAPHMLGLVAGWGISNPNVTVDEIISSGTRTLSDVLQYVKLPVVPHAECKTSYESRSGNYSVTENMFCAGYYEGGKDTCLGDSGGAFVIFDDLSQRWVVQGLVSWGGPEECGSKQVYGVYTKVSNYVDWVWEQMGLPQSVVEPQVER

SEQ ID NO: 9 - DNA, 2852 bp, homo sapiens
tggcgatacattcacacaggaacagctatgccatgtttacgaattccggttttgaaaaaactttcgttgacagttacacaaagggtcacttcctccccagcgacacatgggcctctcaaaggagaggagggagtaagtcccacggtagggccagtggttgctccctgggttttggaatcatttctgcggagctttcaaggccagaccctgggcttagggtcgagactttatagcagtgacagccagacccagcaagatggctgcgaccgtgaaaccctgggcggcgatccgggtgcgcatcatgagctgagagcgctggctgttgccccggtggaaggagtagaggccgtaggtgagggcggccgccgtggccaggcaacctatgggtaccaccgggttctcgcgggcaagtcaagctgggaggaccaaggccgggcagccgggagcacccaaggcaggaaaatgaggtggctgcttctctattatgctctgtgcttctccctgtcaaaggcttcagcccacaccgtggagctaaacaatatgtttggccagatccagtcgcctggttatccagactcctatcccagtgattcagaggtgacttggaatatcactgtcccagatgggtttcggatcaagctttacttcatgcacttcaacttggaatcctcctacctttgtgaatatgactatgtgaaggtagaaactgaggaccaggtgctggcaaccttctgtggcagggagaccacagacacagagcagactcccggccaggaggtggtcctctcccctggctccttcatgtccatcactttccggtcagatttctccaatgaggagcgtttcacaggctttgatgcccactacatggctgtggatgtggacgagtgcaaggagagggaggacgaggagctgtcctgtgaccactactgccacaactacattggcggctactactgctcctgccgcttcggctacatcctccacacagacaacaggacctgccgagtggagtgcagtgacaacctcttcactcaaaggactggggtgatcaccagccctgacttcccaaacccttaccccaagagctctgaatgcctgtataccatcgagctggaggagggtttcatggtcaacctgcagtttgaggacatatttgacattgaggaccatcctgaggtgccctgcccctatgactacatcaagatcaaagttggtccaaaagttttggggcctttctgtggagagaaagccccagaacccatcagcacccagagccacagtgtcctgatcctgttccatagtgacaactcgggagagaaccggggctggaggctctcatacagggctgcaggaaatgagtgcccagagctacagcctcctgtccatgggaaaatcgagccctcccaagccaagtatttcttcaaagaccaagtgctcgtcagctgtgacacaggctacaaagtgctgaaggataatgtggagatggacacattccagattgagtgtctgaaggatgggacgtggagtaacaagattcccacctgtaaaattgtagactgtagagccccaggagagctggaacacgggctgatcaccttctctacaaggaacaacctcaccacatacaagtctgagatcaaatactcctgtcaggagccctattacaagatgctcaacaataacacaggtatatatacctgttctgcccaaggagtctggatgaataaagtattggggagaagcctacccacctgccttccagtgtgtgggctccccaagttctcccggaagctgatggccaggatcttcaatggacgcccagcccagaaaggcaccactccctggattgccatgctgtcacacctgaatgggcagcccttctgcggaggctcccttctaggctccagctggatcgtgaccgccgcacactgcctccaccagtcactcgatccgaaagatccgaccctacgtgattcagacttgctcagcccttctgacttcaaaatcatcctgggcaagcattggaggctccggtcagatgaaaatgaacagcatctcggcgtaaaacacaccactctccaccccaagtatgatcccaacacattcgagaatgacgtggctctggtggagctgttggagagcccagtgctgaatgccttcgtgatgcccatctgtctgcctgagggaccccagcaggaaggagccatggtcatcgtcagcggctggggaaagcagttcttgcaaaggttcccagagaccctgatggagattgaaatcccgattgttgaccacagcacctgccagaaggcttatgccccgctgaagaagaaagtgaccagggacatgatctgtgctggggagaaggaagggggaaaggacgcctgttcgggtgactctggaggccccatggtgaccctgaatagagaaagaggccagtggtacctggtgggcactgtgtcctggggtgatgactgtgggaagaaggaccgctacggagtatactcttacatccaccacaacaaggactggatccagagggtcaccggagtgaggaactgaatttggctcctcagccccagcaccaccagctgtgggcagtcagtagcagaggacgatcctccgatgaaagcagccatttctcctttccttcctcccatcccccctccttcggcctatccattactgggcaatagagcaggtatcttcacccccttttcactctctttaaagagatggagcaagagagtggtcagaacacaggccgaatccaggctctatcacttactagttttcagttctgggcaggtgacttcatctcttcgaacttcagtttcttcataagatggaaa

SEQ ID NO: 10 - protein, 699 aa, homo sapiens
MRWLLLYYALCFSLSKASAHTVELNNMFGQIQSPGYPDSYPSDSEVTWNITVPDGFRIKLYFMHFNLESSYLCEYDYVKVETEDQVLATFCGRETTDTEQTPGQEVVLSPGSFMSITFRSDFSNEERFTGFDAHYMAVDVDECKEREDEELSCDHYCHNYIGGYYCSCRFGYILHTDNRTCRVECSDNLFTQRTGVITSPDFPNPYPKSSECLYTIELEEGFMVNLQFEDIFDIEDHPEVPCPYDYIKIKVGPKVLGPFCGEKAPEPISTQSHSVLILFHSDNSGENRGWRLSYRAAGNECPELQPPVHGKIEPSQAKYFFKDQVLVSCDTGYKVLKDNVEMDTFQIECLKDGTWSNKIPTCKIVDCRAPGELEHGLITFSTRNNLTTYKSEIKYSCQEPYYKMLNNNTGIYTCSAQGVWMNKVLGRSLPTCLPVCGLPKFSRKLMARIFNGRPAQKGTTPWIAMLSHLNGQPFCGGSLLGSSWIVTAAHCLHQSLDPKDPTLRDSDLLSPSDFKIILGKHWRLRSDENEQHLGVKHTTLHPKYDPNTFENDVALVELLESPVLNAFVMPICLPEGPQQEGAMVIVSGWGKQFLQRFPETLMEIEIPIVDHSTCQKAYAPLKKKVTRDMICAGEKEGGKDACSGDSGGPMVTLNRERGQWYLVGTVSWGDDCGKKDRYGVYSYIHHNKDWIQRVTGVRN

SEQ ID NO: 11 - protein, 380 aa, homo sapiens
MRWLLLYYALCFSLSKASAHTVELNNMFGQIQSPGYPDSYPSDSEVTWNITVPDGFRIKLYFMHFNLESSYLCEYDYVKVETEDQVLATFCGRETTDTEQTPGQEVVLSPGSFMSITFRSDFSNEERFTGFDAHYMAVDVDECKEREDEELSCDHYCHNYIGGYYCSCRFGYILHTDNRTCRVECSDNLFTQRTGVITSPDFPNPYPKSSECLYTIELEEGFMVNLQFEDIFDIEDHPEVPCPYDYIKIKVGPKVLGPFCGEKAPEPISTQSHSVLILFHSDNSGENRGWRLSYRAAGNECPELQPPVHGKIEPSQAKYFFKDQVLVSCDTGYKVLKDNVEMDTFQIECLKDGTWSNKIPTCKKNEIDLESELKSEQVTE

SEQ ID NO: 12 - DNA, 2091 bp, rattus
tggcacacaatgaggctactgatcgtcctgggtctgctttggagtttggtggccacacttttgggctccaagtggcctgagcctgtattcgggcgcctggtgtccctggccttcccagagaagtatggcaaccatcaggatcgatcctggacgctgactgcaccccctggcttccgcctgcgcctctacttcacccacttcaacctggaactctcttaccgctgcgagtatgactttgtcaagttgacctcagggaccaaggtgctagccacgctgtgtgggcaggagagtacagatactgagcgggcacctggcaatgacaccttctactcactgggtcccagcctaaaggtcaccttccactccgactactccaatgagaagccattcacaggatttgaggccttctatgcagcggaggatgtggatgaatgcagaacatccctgggagactcagtcccttgtgaccattattgccacaactacctgggcggctactactgctcctgccgagtgggctacattctgcaccagaacaagcatacctgctcagccctttgttcaggccaggtgttcactgggaggtctggctttctcagtagccctgagtacccacagccataccccaaactctccagctgcgcctacaacatccgcctggaggaaggcttcagtatcaccctggacttcgtggagtcctttgatgtggagatgcaccctgaagcccagtgcccctacgactccctcaagattcaaacagacaagagggaatacggcccgttttgtgggaagacgctgccccccaggattgaaactgacagcaacaaggtgaccattacctttaccaccgacgagtcagggaaccacacaggctggaagatacactacacaagcacagcacagccctgccctgatccaacggcgccacctaatggtcacatttcacctgtgcaagccacgtatgtcctgaaggacagcttttctgtcttctgcaagactggcttcgagcttctgcaaggttctgtccccctgaagtcattcactgctgtctgtcagaaagatggatcttgggaccggccgataccagagtgcagcattattgactgtggccctcccgatgacctacccaatggccacgtggactatatcacaggccctgaagtgaccacctacaaagctgtgattcagtacagctgtgaagagactttctacacaatgagcagcaatggtaaatatgtgtgtgaggctgatggattctggacgagctccaaaggagaaaaatccctcccggtttgcaagcctgtctgtggactgtccacacacacttcaggaggccgtataattggaggacagcctgcaaagcctggtgactttccttggcaagtcttgttactgggtgaaactacagcagcaggtgctcttatacatgacgactgggtcctaacagcggctcatgctgtatatgggaaaacagaggcgatgtcctccctggacatccgcatgggcatcctcaaaaggctctccctcatttacactcaagcctggccagaggctgtctttatccatgaaggctacactcacggagctggttttgacaatgatatagcactgattaaactcaagaacaaagtcacaatcaacagaaacatcatgccgatttgtctaccaagaaaagaagctgcatccttaatgaaaacagacttcgttggaactgtggctggctgggggttaacccagaaggggtttcttgctagaaacctaatgtttgtggacataccaattgttgaccaccaaaaatgtgctactgcgtatacaaagcagccctacccaggagcaaaagtgactgttaacatgctctgtgctggcctagaccgcggtggcaaggacagctgcagaggtgacagcggaggggcattagtgtttctagacaatgaaacacagagatggtttgtgggaggaatagtttcctggggttctattaactgtggggggtcagaacagtatggggtctacacgaaagtcacgaactatattccctggattgagaacataataaataatttctaatttgcaaaaaaaaaaaaaaaaaaa

SEQ ID NO: 13 - protein, 685 aa, rattus
MRLLIVLGLLWSLVATLLGSKWPEPVFGRLVSLAFPEKYGNHQDRSWTLTAPPGFRLRLYFTHFNLELSYRCEYDFVKLTSGTKVLATLCGQESTDTERAPGNDTFYSLGPSLKVTFHSDYSNEKPFTGFEAFYAAEDVDECRTSLGDSVPCDHYCHNYLGGYYCSCRVGYILHQNKHTCSALCSGQVFTGRSGFLSSPEYPQPYPKLSSCAYNIRLEEGFSITLDFVESFDVEMHPEAQCPYDSLKIQTDKREYGPFCGKTLPPRIETDSNKVTITFTTDESGNHTGWKIHYTSTAQPCPDPTAPPNGHISPVQATYVLKDSFSVFCKTGFELLQGSVPLKSFTAVCQKDGSWDRPIPECSIIDCGPPDDLPNGHVDYITGPEVTTYKAVIQYSCEETFYTMSSNGKYVCEADGFWTSSKGEKSLPVCKPVCGLSTHTSGGRIIGGQPAKPGDFPWQVLLLGETTAAGALIHDDWVLTAAHAVYGKTEAMSSLDIRMGILKRLSLIYTQAWPEAVFIHEGYTHGAGFDNDIALIKLKNKVTINRNIMPICLPRKEAASLMKTDFVGTVAGWGLTQKGFLARNLMFVDIPIVDHQKCATAYTKQPYPGAKVTVNMLCAGLDRGGKDSCRGDSGGALVFLDNETQRWFVGGIVSWGSINCGGSEQYGVYTKVTNYIPWIENIINNF

SEQ ID NO: 14 - DNA, 354 bp, artificial sequence
  Synthetic
caggtcaccttgaaggagtctggtcctgtgctggtgaaacccacagagaccctcacgctgacctgcaccgtctctgggttctcactcagcaggggtaaaatgggtgtgagctggatccgtcagcccccagggaaggccctggagtggcttgcacacattttttcgagtgacgaaaaatcctacaggacatcgctgaagagcaggctcaccatctccaaggacacctccaaaaaccaggtggtccttacaatgaccaacatggaccctgtggacacagccacgtattactgtgcacggatacgacgtggaggaattgactactggggccagggaaccctggtcactgtctcctca

SEQ ID NO: 15 - protein, 118 aa, artificial sequence
  Synthetic
QVTLKESGPVLVKPTETLTLTCTVSGFSLSRGKMGVSWIRQPPGKALEWLAHIFSSDEKSYRTSLKSRLTISKDTSKNQVVLTMTNMDPVDTATYYCARIRRGGIDYWGQGTLVTVSS

SEQ ID NO: 16 - protein, 121 aa, artificial sequence
  Synthetic
QVQLQQSGPGLVKPSQTLSLTCAISGDSVSSTSAAWNWIRQSPSRGLEWLGRTYYRSKWYNDYAVSVKSRITINPDTSKNQFSLQLNSVTPEDTAVYYCARDPFGVPFDIWGQGTMVTVSS

SEQ ID NO: 17 - protein, 106 aa, artificial sequence
  Synthetic
QPVLTQPPSLSVSPGQTASITCSGEKLGDKYAYWYQQKPGQSPVLVMYQDKQRPSGIPERFSGSNSGNTATLTISGTQAMDEADYYCQAWDSSTAVFGGGTKLTVL

SEQ ID NO: 18 - DNA, 324 bp, artificial sequence
  Synthetic
tcctatgagctgatacagccaccctcggtgtcagtggccccaggacagacggccaccattacctgtgcgggagacaaccttgggaagaaacgtgtgcactggtaccagcagaggccaggccaggcccctgtgttggtcatctatgatgatagcgaccggccctcagggatccctgaccgattctctgcctccaactctgggaacacggccaccctgaccatcactaggggcgaagccggggatgaggccgactattattgtcaggtgtgggacattgctactgatcatgtggtcttcggcggagggaccaagctcaccgtccta

SEQ ID NO: 19 - protein, 120 aa, artificial sequence
  Synthetic
SYELIQPPSVSVAPGQTATITCAGDNLGKKRVHWYQQRPGQAPVLVIYDDSDRPSGIPDRFSASNSGNTATLTITRGEAGDEADYYCQVWDIATDHVVFGGGTKLTVLAAAGSEQKLISE

SEQ ID NO: 20 - protein, 262 aa, artificial sequence
  Synthetic
QVQLQQSGPGLVKPSQTLSLTCAISGDSVSSTSAAWNWIRQSPSRGLEWLGRTYYRSKWYNDYAVSVKSRITINPDTSKNQFSLQLNSVTPEDTAVYYCARDPFGVPFDIWGQGTMVTVSSKLSGSASAPKLEEGEFSEARVSYELIQPPSVSVAPGQTATITCAGDNLGKKRVHWYQQRPGQAPVLVIYDDSDRPSGIPDRFSASNSGNTATLTITRGEAGDEADYYCQVWDIATDHVVFGGGTKLTVLAAAGSEQKLISE

SEQ ID NO: 21 - protein, 245 aa, artificial sequence
  Synthetic
QVTLKESGPVLVKPTETLTLTCTVSGFSLSRGKMGVSWIRQPPGKALEWLAHIFSSDEKSYRTSLKSRLTISKDTSKNQVVLTMTNMDPVDTATYYCARIRRGGIDYWGQGTLVTVSSKLSGSASAPKLEEGEFSEARVQPVLTQPPSLSVSPGQTASITCSGEKLGDKYAYWYQQKPGQSPVLVMYQDKQRPSGIPERFSGSNSGNTATLTISGTQAMDEADYYCQAWDSSTAVFGGGTKLTVL

SEQ ID NO: 22 - DNA, 750 bp, artificial sequence
  Synthetic
caggtacagctgcagcagtcaggtccaggactggtgaagccctcgcagaccctctcactcacctgtgccatctccggggacagtgtctctagcaccagtgctgcttggaactggatcaggcagtccccatcgagaggccttgagtggctgggaaggacatactacaggtccaagtggtataatgattatgcagtatctgtgaaaagtcgaataaccatcaacccagacacatccaagaaccagttctccctgcagctgaactctgtgactcccgaggacacggctgtgtattactgtgcaagagatcctttcggggtaccttttgatatctggggccaagggacaatggtcaccgtctcttcaaagctttcagggagtgcatccgccccaaaacttgaagaaggtgaattttcagaagcacgcgtatcctatgagctgatacagccaccctcggtgtcagtggccccaggacagacggccaccattacctgtgcgggagacaaccttgggaagaaacgtgtgcactggtaccagcagaggccaggccaggcccctgtgttggtcatctatgatgatagcgaccggccctcagggatccctgaccgattctctgcctccaactctgggaacacggccaccctgaccatcactaggggcgaagccggggatgaggccgactattattgtcaggtgtgggacattgctactgatcatgtggtcttcggcggagggaccaagctcaccgtccta

SEQ ID NO: 23 - DNA, 735 bp, artificial sequence
  Synthetic
  misc_feature (663)..(663): n is a, c, g, or t
caggtcaccttgaaggagtctggtcctgtgctggtgaaacccacagagaccctcacgctgacctgcaccgtctctgggttctcactcagcaggggtaaaatgggtgtgagctggatccgtcagcccccagggaaggccctggagtggcttgcacacattttttcgagtgacgaaaaatcctacaggacatcgctgaagagcaggctcaccatctccaaggacacctccaaaaaccaggtggtccttacaatgaccaacatggaccctgtggacacagccacgtattactgtgcacggatacgacgtggaggaattgactactggggccagggaaccctggtcactgtctcctcaaagctttcagggagtgcatccgccccaaaacttgaagaaggtgaattttcagaagcacgcgtacagccagtgctgactcagcccccctcactgtccgtgtccccaggacagacagccagcatcacctgctctggagagaaattgggggataaatatgcttactggtatcagcagaagccaggccagtcccctgtgttggtcatgtatcaagataaacagcggccctcagggatccctgagcgattctctggctccaactctgggaacacagccactctgaccatcagcgggacccaggctatggatgangctgactattactgtcaggcgtgggacagcagcactgcggtattcggcggagggaccaagctgaccgtccta

SEQ ID NO: 24 - protein, 125 aa, artificial sequence
  Synthetic
AVTLDESGGGLQTPGGALSLVCKASGFTFSSNAMGWVRQAPGKGLEWVAGIDDDGSGTRYAPAVKGRATISRDNGQSTLRLQLNNLRAEDTGTYYCTKCAYSSGCDYEGGYIDAWGHGTEVIVSS

SEQ ID NO: 25 - protein, 118 aa, artificial sequence
  Synthetic
AVTLDESGGGLQTPGGGLSLVCKASGFTFSSYAMGWMRQAPGKGLEYVAGIRSDGSFTLYATAVKGRATISRDNGQSTVRLQLNNLRAEDTATYFCTRSGNVGDIDAWGHGTEVIVSS

SEQ ID NO: 26 - protein, 128 aa, artificial sequence
  Synthetic
AVTLDESGGGLQTPGGGLSLVCKASGFDFSSYQMNWIRQAPGKGLEFVAAINRFGNSTGHGAAVKGRVTISRDDGQSTVRLQLSNLRAEDTATYYCAKGVYGYCGSYSCCGVDTIDAWGHGTEVIVSS

SEQ ID NO: 27 - protein, 107 aa, artificial sequence
  Synthetic
ALTQPASVSANLGGTVKITCSGGGSYAGSYYYGWYQQKSPGSAPVTVIYDNDKRPSDIPSRFSGSLSGSTNTLTITGVRADDEAVYFCGSADNSGAAFGAGTTLTVL

SEQ ID NO: 28 - protein, 108 aa, artificial sequence
  Synthetic
ALTQPASVSANPGETVKITCSGGYSGYAGSYYYGWYQQKAPGSAPVTLIYYNNKRPSDIPSRFSGSLSGSTNTLTITGVRADDEAVYFCGSADNSGAAFGAGTTLTVL

SEQ ID NO: 29 - protein, 107 aa, artificial sequence
  Synthetic
ALTQPASVSANPGETVKITCSGGGSYAGSYYYGWYQQKAPGSAPVTLIYYNNKRPSDIPSRFSGSLSGSTNTLTITGVRADDEAVYFCGSADNSGAAFGAGTTLTVL

SEQ ID NO: 30 - protein, 126 aa, artificial sequence
  Synthetic
AVTLDESGGGLQTPGGALSLVCKASGFTFSSYAMHWVRQAPGKGLEWVAGIYKSGAGTNYAPAVKGRATISRDNGQSTVRLQLNNLRAEDTGTYYCAKTTGSGCSSGYRAEYIDAWGHGTEVIVSS

SEQ ID NO: 31 - protein, 107 aa, artificial sequence; identical to SEQ ID NO: 29
  Synthetic

SEQ ID NO: 32 - protein, 126 aa, artificial sequence
  Synthetic
AVTLDESGGGLQTPGGALSLVCKASGFTFSSYDMVWVRQAPGKGLEFVAGISRNDGRYTEYGSAVKGRATISRDNGQSTVRLQLNNLRAEDTATYYCARDAGGSAYWFDAGQIDAWGHGTEVIVSS

SEQ ID NO: 33 - protein, 107 aa, artificial sequence; identical to SEQ ID NO: 29
  Synthetic

SEQ ID NO: 34 - protein, 36 aa, artificial sequence
  Synthetic
LEVTCEPGTTFKDKCNTCRCGSDGKSAFCTRKLCYQ

SEQ ID NO: 35 - protein, 36 aa, artificial sequence
  Synthetic
LEVTCEPGTTFKDKCNTCRCGSDGKSAVCTKLWCNQ

SEQ ID NO: 36 - skipped
  Unknown

SEQ ID NO: 37 - protein, 12 aa, artificial sequence
  Synthetic
GTGGGSGSSSRS

SEQ ID NO: 38 - protein, 10 aa, artificial sequence
  Synthetic
GTGGGSGSSS

SEQ ID NO: 39 - skipped
  Unknown

SEQ ID NO: 40 - protein, 275 aa, artificial sequence
  Synthetic
LEVTCEPGTTFKDKCNTCRCGSDGKSAFCTRKLCYQGTGGGSGSSSRSDKTHTCPPCPAPELLGGPSVFLFPPKPKDTLMISRTPEVTCVVVDVSHEDPEVKFNWYVDGVEVHNAKTKPREEQYNSTYRVVSVLTVLHQDWLNGKEYKCKVSNKALPAPIEKTISKAKGQPREPQVYTLPPSREEMTKNQVSLTCLVKGFYPSDIAVEWESNGQPENNYKTTPPVLDSDGSFFLYSKLTVDKSRWQQGNVFSCSVMHEALHNHYTQKSLSLSPGK

SEQ ID NO: 41 - skipped
  Unknown

SEQ ID NO: 42 - protein, 275 aa, artificial sequence
  Synthetic
LEVTCEPGTTFKDKCNTCRCGSDGKSAVCTKLWCNQGTGGGSGSSSRSDKTHTCPPCPAPELLGGPSVFLFPPKPKDTLMISRTPEVTCVVVDVSHEDPEVKFNWYVDGVEVHNAKTKPREEQYNSTYRVVSVLTVLHQDWLNGKEYKCKVSNKALPAPIEKTISKAKGQPREPQVYTLPPSREEMTKNQVSLTCLVKGFYPSDIAVEWESNGQPENNYKTTPPVLDSDGSFFLYSKLTVDKSRWQQGNVFSCSVMHEALHNHYTQKSLSLSPGK